European Patent Application EP 4 190 339 A1, published June 7, 2023. Title: A MODULATABLE SWITCH FOR SELECTION OF DONOR MODIFIED CELLS. Applicant: CSL Gene Therapy Pty Ltd. The sequence listing filed with the application follows.

SEQUENCE LISTING (1 sequence)

SEQ ID NO: 1 - RNA, 92 nt, synthetic construct
  source 1..92: mol_type = other RNA; note = Synthetic: shRNA to knockout HPRT
aggatatgcccttgactatttgtccgacatagtcaagggcatatcctcctatacgggaactgataaacaggctgtatcagttcccgtatagg